European Patent Specification EP 3 460 063 B1, published March 13, 2024. Title: Methods and Compositions for the Targeted Modification of a Genome. Applicant: Frendewey, David Auerbach, Wojtek Lai, Ka-Man Venus Mujica, Alexander O. Lee, Jeffrey D. Droguett, Gustavo Trzaska, Sean Hunt, Charleen Gagliardi, Anthony Kuno, Junko Valenzuela, David M. Yancopoulos, George D. The sequence listing filed with the application follows.

SEQUENCE LISTING (94 sequences)

SEQ ID NO: 1 - DNA, 23 bp, Artificial Sequence
  a genomic target sequence that is linked to a guide RNA (gRNA)
  misc_feature 2, 3, 4, 5, 6, 7, 8, 9, 10, 11, 12, 13, 14, 15, 16, 17, 18,19, 20, 21: n = A,T,C or G
gnnnnnnnnnnnnnnnnnnnngg

SEQ ID NO: 2 - RNA, 80 nt, Artificial Sequence
  a guide RNA (gRNA)
guuuuagagcuagaaauagcaaguuaaaauaaggcuaguccguuaucaacuugaaaaaguggcaccgagucggugcuuuu

SEQ ID NO: 3 - RNA, 42 nt, Artificial Sequence
  a guide RNA (gRNA)
guuuuagagcuagaaauagcaaguuaaaauaaggcuaguccg

SEQ ID NO: 4 - RNA, 30 nt, Artificial Sequence
  a crRNA
guuuuagagcuagaaauagcaaguuaaaau

SEQ ID NO: 5 - RNA, 33 nt, Artificial Sequence
  a crRNA
guuuuagagcuagaaauagcaaguuaaaauaag

SEQ ID NO: 6 - RNA, 26 nt, Artificial Sequence
  a crRNA
gaguccgagcagaagaagaaguuuua

SEQ ID NO: 7 - RNA, 12 nt, Artificial Sequence
  a tracrRNA
aaggcuaguccg

SEQ ID NO: 8 - RNA, 50 nt, Artificial Sequence
  a tracrRNA
aaggcuaguccguuaucaacuugaaaaaguggcaccgagucggugcuuuu

SEQ ID NO: 9 - protein, 203 aa, Mus Musculus [sequence omitted]

SEQ ID NO: 10 - DNA, 15 bp, Artificial Sequence
  ZFN1a binding site
caggccctgaaccgc

SEQ ID NO: 11 - DNA, 6 bp, Artificial Sequence
  ZFN1 cutting site
ttctgg

SEQ ID NO: 12 - DNA, 16 bp, Artificial Sequence
  ZFN1b binding  site
gattacctgcgctggg

SEQ ID NO: 13 - DNA, 15 bp, Artificial Sequence
  ZF21a binding  site
ttcaccctccgcacc

SEQ ID NO: 14 - DNA, 7 bp, Artificial Sequence
  ZFN2 cutting  site
tgctgag

SEQ ID NO: 15 - DNA, 18 bp, Artificial Sequence
  ZF21b binding site
tatccagatccaggggtt

SEQ ID NO: 16 - protein, 9 aa, Artificial Sequence
  conserved domain of a family of homing nucleases
LAGLIDADG

SEQ ID NO: 17 - DNA, 15 bp, Artificial Sequence
  ZFN1a binding site
caggccctgaaccgc

SEQ ID NO: 18 - DNA, 6 bp, Artificial Sequence
  ZFN1 cutting site
ttctgg

SEQ ID NO: 19 - DNA, 16 bp, Artificial Sequence
  ZFN1b binding site
gattacctgcgctggg

SEQ ID NO: 20 - protein, 369 aa, Homo sapiens
MLKPSLPFTSLLFLQLPLLGVGLNTTILTPNGNEDTTADFFLTTMPTDSLSVSTLPLPEVQCFVFNVEYMNCTWNSSSEPQPTNLTLHYWYKNSDNDKVQKCSHYLFSEEITSGCQLQKKEIHLYQTFVVQLQDPREPRRQATQMLKLQNLVIPWAPENLTLHKLSESQLELNWNNRFLNHCLEHLVQYRTDWDHSWTEQSVDYRHKFSLPSVDGQKRYTFRVRSRFNPLCGSAQHWSEWSHPIHWGSNTSKENPFLFALEAVVISVGSMGLIISLLCVYFWLERTMPRIPTLKNLEDLVTEYHGNFSAWSGVSKGLAESLQPDYSERLCLVSEIPPKGGALGEGPGASPCNQHSPYWAPPCYTLKPET

SEQ ID NO: 21 - protein, 368 aa, Rattus norvegicus
MLKPLLPSRSFLLLQLLLLRVGWSSKVLMSSGNEDTKSDLLLTSMDLKHLSVPTLPLPEVQCFVFNVEYMNCTWNSSSEPQPTNLTMHYRYKGSDNNTFQECSHYLFSKEITSGCQIQKEDIQLYQTFVVQLQDPQKPQRRAEQKLNLQNLVIPWAPENLTLYNLSESQVELRWKSRYIERCLQYLVQYRSNRDRSWTEQIVDHEPRFSLPSVDEQKLYTFRVRSRFNPICGSTQQWSKWSQPIHWGSHTAEENPSLFALEAVLIPVGTMGLIITLIFVYCWLERMPRIPAIKNLEDLVTEYHGNFSAWSGVSKGLTESLQPDYSERFCHVSEIPPKGGALGEGPGGSPCSLHSPYWPPPCYSLKPEA

SEQ ID NO: 22 - protein, 368 aa, Artificial Sequence
  chimeric IL-2 receptor gamma comprising the rat IL-2 receptor gamma protein having the ecto domain of IL-2 gamma receptor from human
MLKPSLPFTSLLFLQLPLLGVGLNTTILTPNGNEDTTADFFLTTMPTDSLSVSTLPLPEVQCFVFNVEYMNCTWNSSSEPQPTNLTLHYWYKNSDNDKVQKCSHYLFSEEITSGCQLQKKEIHLYQTFVVQLQDPREPRRQATQMLKLQNLVIPWAPENLTLHKLSESQLELNWNNRFLNHCLEHLVQYRTDWDHSWTEQSVDYRHKFSLPSVDGQKRYTFRVRSRFNPLCGSAQHWSEWSHPIHWGSNTSKENPFLFALEAVLIPVGTMGLIITLIFVYCWLERMPRIPAIKNLEDLVTEYHGNFSAWSGVSKGLTESLQPDYSERFCHVSEIPPKGGALGEGPGGSPCSLHSPYWPPPCYSLKPEA

SEQ ID NO: 23 - DNA, 23 bp, Artificial Sequence
  a genomic target sequence that is linked to a guide RNA (gRNA)
  misc_feature (2)...(21): n= A, T, C or G
  misc_feature (0)...(0): n can be from 1-20 nucleotides
gnnnnnnnnnnnnnnnnnnnngg

SEQ ID NO: 24 - DNA, 20 bp, Artificial Sequence
  a guide sequence
gggaacccacagcatactcc

SEQ ID NO: 25 - DNA, 20 bp, Artificial Sequence
  a guide sequence
gaatcatgcacggctacccc

SEQ ID NO: 26 - DNA, 20 bp, Artificial Sequence
  a guide sequence
tgctcctatggggaggcgcg

SEQ ID NO: 27 - DNA, 20 bp, Artificial Sequence
  a guide sequence
cttggataacattgataccc

SEQ ID NO: 28 - DNA, 20 bp, Artificial Sequence
  a guide sequence
ggggcagagcccttatatca

SEQ ID NO: 29 - DNA, 20 bp, Artificial Sequence
  a guide sequence
tcgctcacattaatccctag

SEQ ID NO: 30 - DNA, 20 bp, Artificial Sequence
  a guide sequence
gtactggggaatcggtggtc

SEQ ID NO: 31 - DNA, 20 bp, Artificial Sequence
  a guide sequence
cacgcactccaaatttatcc

SEQ ID NO: 32 - DNA, 20 bp, Artificial Sequence
  a guide sequence
ctaagtgtgtatcagtacat

SEQ ID NO: 33 - DNA, 20 bp, Artificial Sequence
  a guide sequence
tgccctgcacaataagcgca

SEQ ID NO: 34 - DNA, 20 bp, Artificial Sequence
  a guide sequence
actcattgaaacgttatggc

SEQ ID NO: 35 - DNA, 20 bp, Artificial Sequence
  a guide sequence
agtaagggtggattaaattc

SEQ ID NO: 36 - DNA, 20 bp, Artificial Sequence
  a guide sequence
gccatctagattcatgtaac

SEQ ID NO: 37 - DNA, 20 bp, Artificial Sequence
  a guide sequence
gactagaaatgttctgcacc

SEQ ID NO: 38 - DNA, 20 bp, Artificial Sequence
  a guide sequence
tgaaccaattgtgtagcctt

SEQ ID NO: 39 - DNA, 20 bp, Artificial Sequence
  a guide sequence
aatagtggtaaagcaccatg

SEQ ID NO: 40 - DNA, 20 bp, Artificial Sequence
  a guide sequence
gtgtgctaaggatcgaagtc

SEQ ID NO: 41 - DNA, 20 bp, Artificial Sequence
  a guide sequence
caccgagatgcttgggtatt

SEQ ID NO: 42 - DNA, 20 bp, Artificial Sequence
  a guide sequence
tgtaaccgccctgaatgacc

SEQ ID NO: 43 - DNA, 20 bp, Artificial Sequence
  a guide sequence
aaaagggcatcataaatccc

SEQ ID NO: 44 - DNA, 20 bp, Artificial Sequence
  a guide sequence
tcaaaaatagtcatacacct

SEQ ID NO: 45 - DNA, 20 bp, Artificial Sequence
  a guide sequence
ggtctctagtacattgtaga

SEQ ID NO: 46 - DNA, 20 bp, Artificial Sequence
  a guide sequence
atcacaaaccagttaaccgg

SEQ ID NO: 47 - DNA, 20 bp, Artificial Sequence
  a guide sequence
tttcagacgagccgacccgg

SEQ ID NO: 48 - DNA, 20 bp, Artificial Sequence
  a guide sequence
ctgtcaacagtgccgcgttt

SEQ ID NO: 49 - DNA, 20 bp, Artificial Sequence
  a guide sequence
tgtgtgtcatagcgatgtcg

SEQ ID NO: 50 - DNA, 20 bp, Artificial Sequence
  a guide sequence
aacaggtaccctatcctcac

SEQ ID NO: 51 - DNA, 20 bp, Artificial Sequence
  a guide sequence
tcgtggttgcatgcgcactg

SEQ ID NO: 52 - DNA, 20 bp, Artificial Sequence
  a guide sequence
ggcccggacctagtctctct

SEQ ID NO: 53 - DNA, 20 bp, Artificial Sequence
  a guide sequence
agtctgtaaagttagcagtc

SEQ ID NO: 54 - DNA, 20 bp, Artificial Sequence
  a guide sequence
ggtggtggtgctgacggaca

SEQ ID NO: 55 - DNA, 20 bp, Artificial Sequence
  a guide sequence
tatgagatcaacactcgcta

SEQ ID NO: 56 - DNA, 20 bp, Artificial Sequence
  a guide sequence
ccaaggacttccccacgtta

SEQ ID NO: 57 - DNA, 20 bp, Artificial Sequence
  a guide sequence
tgcttcccttatgcaagatt

SEQ ID NO: 58 - DNA, 20 bp, Artificial Sequence
  a guide sequence
ttaggtaccctatttgaata

SEQ ID NO: 59 - DNA, 20 bp, Artificial Sequence
  a guide sequence
tgcagtgggtgacaggtcca

SEQ ID NO: 60 - DNA, 20 bp, Artificial Sequence
  a guide sequence
agggttatactgacgttgtg

SEQ ID NO: 61 - DNA, 20 bp, Artificial Sequence
  a guide sequence
tgtctttcaaggagggctac

SEQ ID NO: 62 - DNA, 20 bp, Artificial Sequence
  a guide sequence
tgatgtgcagtcagacaaag

SEQ ID NO: 63 - DNA, 20 bp, Artificial Sequence
  a guide sequence
tgcactatggttgactatga

SEQ ID NO: 64 - DNA, 20 bp, Artificial Sequence
  a guide sequence
ggaatattctaataggaagt

SEQ ID NO: 65 - DNA, 20 bp, Artificial Sequence
  a guide sequence
aagtgctgtaccattctagc

SEQ ID NO: 66 - DNA, 20 bp, Artificial Sequence
  a guide sequence
taatcaatagacaacctcgt

SEQ ID NO: 67 - DNA, 20 bp, Artificial Sequence
  a guide sequence
tcattcctaatggtattata

SEQ ID NO: 68 - DNA, 20 bp, Artificial Sequence
  a guide sequence
agggtacatagatggcatcg

SEQ ID NO: 69 - DNA, 20 bp, Artificial Sequence
  a guide sequence
ctctttaacaattaccactt

SEQ ID NO: 70 - DNA, 20 bp, Artificial Sequence
  a guide sequence
tgtgggcctttgctgatcac

SEQ ID NO: 71 - DNA, 20 bp, Artificial Sequence
  a guide sequence
aatctatgatcctatggcct

SEQ ID NO: 72 - DNA, 20 bp, Artificial Sequence
  a guide sequence
tgccaatagcagtgacttga

SEQ ID NO: 73 - DNA, 20 bp, Artificial Sequence
  a guide sequence
gggaagaatgggctattgtc

SEQ ID NO: 74 - DNA, 20 bp, Artificial Sequence
  a guide sequence
ggttgtttgtgctgatgacg

SEQ ID NO: 75 - DNA, 20 bp, Artificial Sequence
  a guide sequence
ccgtcctaggccttctacgt

SEQ ID NO: 76 - DNA, 20 bp, Artificial Sequence
  a guide sequence
actagtagacctgaggggtt

SEQ ID NO: 77 - DNA, 20 bp, Artificial Sequence
  a guide sequence
gctccagtgtttaggccttg

SEQ ID NO: 78 - DNA, 20 bp, Artificial Sequence
  a guide sequence
ggcaagctgaaaacgcatgc

SEQ ID NO: 79 - DNA, 20 bp, Artificial Sequence
  a guide sequence
gtagatcgctttccactacc

SEQ ID NO: 80 - DNA, 20 bp, Artificial Sequence
  a guide sequence
gaactccactgctcgtgagc

SEQ ID NO: 81 - DNA, 20 bp, Artificial Sequence
  a guide sequence
ataggtgggcactattgaag

SEQ ID NO: 82 - DNA, 20 bp, Artificial Sequence
  a guide sequence
atgggaaggtttataccagc

SEQ ID NO: 83 - DNA, 20 bp, Artificial Sequence
  a guide sequence
cggtgtaaaaacaacgggaa

SEQ ID NO: 84 - RNA, 20 nt, Artificial Sequence
  a guide sequence
gacccgcagucccagcgucg

SEQ ID NO: 85 - DNA, 20 bp, Artificial Sequence
  a guide sequence
actgagatcaatgaccccga

SEQ ID NO: 86 - DNA, 20 bp, Artificial Sequence
  a guide sequence
gggtcgcccggaacctctac

SEQ ID NO: 87 - DNA, 23 bp, Artificial Sequence
  a guide sequence
gcaggccctgaaccgcttcttgg

SEQ ID NO: 88 - DNA, 23 bp, Artificial Sequence
  a guide sequence
cctgcgctgggtgcagacgcttt

SEQ ID NO: 89 - DNA, 20 bp, Artificial Sequence
  a guide sequence
ccagctacttgctcgtacaa

SEQ ID NO: 90 - DNA, 20 bp, Artificial Sequence
  a guide sequence
cccctcagattcacgtgcgt

SEQ ID NO: 91 - DNA, 23 bp, Artificial Sequence
  a guide sequence
gaagctctttctatacaatctgg

SEQ ID NO: 92 - DNA, 23 bp, Artificial Sequence
  a guide sequence
cccccgaaaggaggagccctagg

SEQ ID NO: 93 - DNA, 56 bp, Rattus norvegicus
ttctgagcctcagccgaccaacctcactatgcactataggtatgagaagggggagg

SEQ ID NO: 94 - DNA, 20 bp, aArtificial Sequence
  a guide sequence
gtatagccctgttacacatt